European Patent Application EP 4 534 094 A1, published April 9, 2025. Title: 락토바실러스 플란타룸 NCHBL-004 균주 또는 이의 배양액을 포함하는 대사성 질환 예방, 치료 또는 개선용 조성물. Applicant: 전남대학교산학협력단. The sequence listing filed with the application follows.

SEQUENCE LISTING (23 sequences)

SEQ ID NO: 1 - DNA, 982 bp, Lactobacillus plantarum
  source 1..982: mol_type = genomic DNA
tgcagtcgaacgaactctggtattgattggtgcttgcatcatgatttacatttgagtgagtggcgaactggtgagtaacacgtgggaaacctgcccagaagcgggggataacacctggaaacagatgctaataccgcataacaacttggaccgcatggtccgagtttgaaagatggcttcggctatcacttttggatggtcccgcggcgtattagctagatggtggggtaacggctcaccatggcaatgatacgtagccgacctgagagggtaatcggccacattgggactgagacacggcccaaactcctacgggaggcagcagtagggaatcttccacaatggacgaaagtctgatggagcaacgccgcgtgagtgaagaagggtttcggctcgtaaaactctgttgttaaagaagaacatatctgagagtaactgttcaggtattgacggtatttaaccagaaagccacggctaactacgtgccagcagccgcggtaatacgtaggtggcaagcgttgtccggatttattgggcgtaaagcgagcgcaggcggttttttaagtctgatgtgaaagccttcggctcaaccgaagaagtgcatcggaaactgggaaacttgagtgcagaagaggacagtggaactccatgtgtagcggtgaaatgcgtagatatatggaagaacaccagtggcgaaggcggctgtctggtctgtaactgacgctgaggctcgaaagtatgggtagcaaacaggattagataccctggtagtccataccgtaaacgatgaatgctaagtgttggagggtttccgcccttcagtgctgcagctaacgcattaagcattccgcctggggagtacggccgcaaggctgaaactcaaaggaattgacgggggcccgcacaagcggtggagcatgtggtttaattcgaagctacgcgaagaaccttaccaggtcttgacatactatgcaaatctaag

SEQ ID NO: 2 - DNA, 20 bp, synthetic construct
  misc_feature 1..20: note = 18S rRNA forward primer
  source 1..20: mol_type = other DNA
aggagctgaagggccacggg

SEQ ID NO: 3 - DNA, 20 bp, synthetic construct
  misc_feature 1..20: note = 18S rRNA reverse primer
  source 1..20: mol_type = other DNA
tgggaacagtgacgcgggtc

SEQ ID NO: 4 - DNA, 20 bp, synthetic construct
  misc_feature 1..20: note = Adiponectin forward primer
  source 1..20: mol_type = other DNA
aggagctgaagggccacggg

SEQ ID NO: 5 - DNA, 20 bp, synthetic construct
  misc_feature 1..20: note = Adiponectin reverse primer
  source 1..20: mol_type = other DNA
tgggaacagtgacgcgggtc

SEQ ID NO: 6 - DNA, 20 bp, synthetic construct
  misc_feature 1..20: note = GLUT4 forward primer
  source 1..20: mol_type = other DNA
acatacctgacagggcaagg

SEQ ID NO: 7 - DNA, 20 bp, synthetic construct
  misc_feature 1..20: note = GLUT4 reverse primer
  source 1..20: mol_type = other DNA
cgcccttagttggtcagaag

SEQ ID NO: 8 - DNA, 23 bp, synthetic construct
  misc_feature 1..23: note = HSL forward primer
  source 1..23: mol_type = other DNA
tggggagctccagtcggaagagg

SEQ ID NO: 9 - DNA, 21 bp, synthetic construct
  misc_feature 1..21: note = HSL reverse primer
  source 1..21: mol_type = other DNA
cattagacagccgccgtgctg

SEQ ID NO: 10 - DNA, 20 bp, synthetic construct
  misc_feature 1..20: note = ATGL forward primer
  source 1..20: mol_type = other DNA
ctcattcgctggctgcggct

SEQ ID NO: 11 - DNA, 20 bp, synthetic construct
  misc_feature 1..20: note = ATGL reverse primer
  source 1..20: mol_type = other DNA
ccccagtgaccagcgctgtg

SEQ ID NO: 12 - DNA, 20 bp, synthetic construct
  misc_feature 1..20: note = CPT1a forward primer
  source 1..20: mol_type = other DNA
accactggccgcatgtcaag

SEQ ID NO: 13 - DNA, 20 bp, synthetic construct
  misc_feature 1..20: note = CPT1a reverse primer
  source 1..20: mol_type = other DNA
agcgagtagcgcatagtcat

SEQ ID NO: 14 - DNA, 22 bp, synthetic construct
  misc_feature 1..22: note = C/EBPa forward primer
  source 1..22: mol_type = other DNA
gaacagcaacgagtaccgggta

SEQ ID NO: 15 - DNA, 20 bp, synthetic construct
  misc_feature 1..20: note = C/EBPa reverse primer
  source 1..20: mol_type = other DNA
ccatggccttgaccaaggag

SEQ ID NO: 16 - DNA, 20 bp, synthetic construct
  misc_feature 1..20: note = PPARr forward primer
  source 1..20: mol_type = other DNA
ggtgaaactctgggagattc

SEQ ID NO: 17 - DNA, 20 bp, synthetic construct
  misc_feature 1..20: note = PPARr reverse primer
  source 1..20: mol_type = other DNA
caaccattgggtcagctctt

SEQ ID NO: 18 - DNA, 23 bp, synthetic construct
  misc_feature 1..23: note = aP2 forward primer
  source 1..23: mol_type = other DNA
acatgatcatcagcgtaaatggg

SEQ ID NO: 19 - DNA, 23 bp, synthetic construct
  misc_feature 1..23: note = aP2 reverse primer
  source 1..23: mol_type = other DNA
tcataacacattccaccaccagc

SEQ ID NO: 20 - DNA, 20 bp, synthetic construct
  misc_feature 1..20: note = TNF-a forward primer
  source 1..20: mol_type = other DNA
cgtcagccgatttgctatct

SEQ ID NO: 21 - DNA, 20 bp, synthetic construct
  misc_feature 1..20: note = TNF-a reverse primer
  source 1..20: mol_type = other DNA
cggactccgcaaagtctaag

SEQ ID NO: 22 - DNA, 23 bp, synthetic construct
  misc_feature 1..23: note = Caspase1 forward primer
  source 1..23: mol_type = other DNA
aggaattctggagcttcaatcag

SEQ ID NO: 23 - DNA, 21 bp, synthetic construct
  misc_feature 1..21: note = Caspase1 reverse primer
  source 1..21: mol_type = other DNA
tggaaatgtgccatcttcttt